European Patent Specification EP 3 811 983 B1, published October 25, 2023. Title: a composition for cell transplantation and a method for cell transplantation. Applicant: KYOTO UNIVERSITY SANYO CHEMICAL INDUSTRIES, LTD. The sequence listing filed with the application follows.

SEQUENCE LISTING (19 sequences)

SEQ ID NO: 1 - protein, 5 aa, Homo sapiens
VPGVG

SEQ ID NO: 2 - protein, 5 aa, Homo sapiens
GVGVP

SEQ ID NO: 3 - protein, 9 aa, Artificial sequence
  Amino acid sequence(X)
GAHGPAGPK

SEQ ID NO: 4 - protein, 6 aa, Artificial sequence
  Amino acid sequence
GAGAGS

SEQ ID NO: 5 - protein, 24 aa, Artificial sequence
  Polypeptide chain(S)
GAGAGSGAGAGSGAGAGSGAGAGS

SEQ ID NO: 6 - protein, 40 aa, Artificial sequence
  Polypeptide chain(X')
GVGVPGVGVPGVGVPGVGVPGKGVPGVGVPGVGVPGVGVP

SEQ ID NO: 7 - protein, 5 aa, Artificial sequence
  Amino acid sequence(X')
GKGVP

SEQ ID NO: 8 - protein, 5 aa, Artificial sequence
  Amino acid sequence(X')
GKGKP

SEQ ID NO: 9 - protein, 5 aa, Artificial sequence
  Amino acid sequence(X')
GKGRP

SEQ ID NO: 10 - protein, 5 aa, Artificial sequence
  Amino acid sequence(X')
GRGRP

SEQ ID NO: 11 - protein, 5 aa, Artificial sequence
  Amino acid sequence(Z)
VAAGY

SEQ ID NO: 12 - protein, 5 aa, Artificial sequence
  Amino acid sequence(Z)
GAAGY

SEQ ID NO: 13 - protein, 33 aa, Artificial sequence
  Amino acid sequence(T)
MDPVVLQRRDWENPGVTQLNRLAAHPPFASDPM

SEQ ID NO: 14 - protein, 12 aa, Artificial sequence
  Polypeptide chain(S)
GAGAGSGAGAGS

SEQ ID NO: 15 - protein, 884 aa, Artificial sequence
  SELP8K
MDPVVLQRRDWENPGVTQLNRLAAHPPFASDPMGAGSGAGAGSGVGVPGVGVPGVGVPGVGVPGKGVPGVGVPGVGVPGVGVPGAGAGSGAGAGSGAGAGSGAGAGSGVGVPGVGVPGVGVPGVGVPGKGVPGVGVPGVGVPGVGVPGAGAGSGAGAGSGAGAGSGAGAGSGVGVPGVGVPGVGVPGVGVPGKGVPGVGVPGVGVPGVGVPGAGAGSGAGAGSGAGAGSGAGAGSGVGVPGVGVPGVGVPGVGVPGKGVPGVGVPGVGVPGVGVPGAGAGSGAGAGSGAGAGSGAGAGSGVGVPGVGVPGVGVPGVGVPGKGVPGVGVPGVGVPGVGVPGAGAGSGAGAGSGAGAGSGAGAGSGVGVPGVGVPGVGVPGVGVPGKGVPGVGVPGVGVPGVGVPGAGAGSGAGAGSGAGAGSGAGAGSGVGVPGVGVPGVGVPGVGVPGKGVPGVGVPGVGVPGVGVPGAGAGSGAGAGSGAGAGSGAGAGSGVGVPGVGVPGVGVPGVGVPGKGVPGVGVPGVGVPGVGVPGAGAGSGAGAGSGAGAGSGAGAGSGVGVPGVGVPGVGVPGVGVPGKGVPGVGVPGVGVPGVGVPGAGAGSGAGAGSGAGAGSGAGAGSGVGVPGVGVPGVGVPGVGVPGKGVPGVGVPGVGVPGVGVPGAGAGSGAGAGSGAGAGSGAGAGSGVGVPGVGVPGVGVPGVGVPGKGVPGVGVPGVGVPGVGVPGAGAGSGAGAGSGAGAGSGAGAGSGVGVPGVGVPGVGVPGVGVPGKGVPGVGVPGVGVPGVGVPGAGAGSGAGAGSGAGAGSGAGAGSGVGVPGVGVPGVGVPGVGVPGKGVPGVGVPGVGVPGVGVPGAGAGSGAGAGSGAGAMDPGRYQDLRSHHHHHH

SEQ ID NO: 16 - protein, 948 aa, Artificial sequence
  SELP0K
MDPVVLQRRDWENPGVTQLNRLAAHPPFASDPMGAGAGSGAGAGSGVGVPGVGVPGVGVPGVGVPGKGVPGVGVPGVGVPGVGVPGAGAGSGAGAGSGVGVPGVGVPGVGVPGVGVPGKGVPGVGVPGVGVPGVGVPGAGAGSGAGAGSGVGVPGVGVPGVGVPGVGVPGKGVPGVGVPGVGVPGVGVPGAGAGSGAGAGSGVGVPGVGVPGVGVPGVGVPGKGVPGVGVPGVGVPGVGVPGAGAGSGAGAGSGVGVPGVGVPGVGVPGVGVPGKGVPGVGVPGVGVPGVGVPGAGAGSGAGAGSGVGVPGVGVPGVGVPGVGVPGKGVPGVGVPGVGVPGVGVPGAGAGSGAGAGSGVGVPGVGVPGVGVPGVGVPGKGVPGVGVPGVGVPGVGVPGAGAGSGAGAGSGVGVPGVGVPGVGVPGVGVPGKGVPGVGVPGVGVPGVGVPGAGAGSGAGAGSGVGVPGVGVPGVGVPGVGVPGKGVPGVGVPGVGVPGVGVPGAGAGSGAGAGSGVGVPGVGVPGVGVPGVGVPGKGVPGVGVPGVGVPGVGVPGAGAGSGAGAGSGVGVPGVGVPGVGVPGVGVPGKGVPGVGVPGVGVPGVGVPGAGAGSGAGAGSGVGVPGVGVPGVGVPGVGVPGKGVPGVGVPGVGVPGVGVPGAGAGSGAGAGSGVGVPGVGVPGVGVPGVGVPGKGVPGVGVPGVGVPGVGVPGAGAGSGAGAGSGVGVPGVGVPGVGVPGVGVPGKGVPGVGVPGVGVPGVGVPGAGAGSGAGAGSGVGVPGVGVPGVGVPGVGVPGKGVPGVGVPGVGVPGVGVPGAGAGSGAGAGSGVGVPGVGVPGVGVPGVGVPGKGVPGVGVPGVGVPGVGVPGAGAGSGAGAGSGVGVPGVGVPGVGVPGVGVPGKGVPGVGVPGVGVPGVGVPGAGAGSGAGAGSGAMDPGRYQDLRSHHHHHH

SEQ ID NO: 17 - protein, 1384 aa, Artificial sequence
  SLP4.1
MDPVVLQRRDWENPGVTQLNRLAAHPPFASDPMGAGAGSGAGAGSGAGAGSGAGAGSGAGAGSGAGAGSGVGVPGVGVPGAGAGSGAGAGSGAGAGSGAGAGSGAGAGSGAGAGSGVGVPGVGVPGAGAGSGAGAGSGAGAGSGAGAGSGAGAGSGAGAGSGVGVPGVGVPGAGAGSGAGAGSGAGAGSGAGAGSGAGAGSGAGAGSGVGVPGVGVPGAGAGSGAGAGSGAGAGSGAGAGSGAGAGSGAGAGSGVGVPGVGVPGAGAGSGAGAGSGAGAGSGAGAGSGAGAGSGAGAGSGVGVPGVGVPGAGAGSGAGAGSGAGAGSGAGAGSGAGAGSGAGAGSGVGVPGVGVPGAGAGSGAGAGSGAGAGSGAGAGSGAGAGSGAGAGSGVGVPGVGVPGAGAGSGAGAGSGAGAGSGAGAGSGAGAGSGAGAGSGVGVPGVGVPGAGAGSGAGAGSGAGAGSGAGAGSGAGAGSGAGAGSGVGVPGVGVPGAGAGSGAGAGSGAGAGSGAGAGSGAGAGSGAGAGSGVGVPGVGVPGAGAGSGAGAGSGAGAGSGAGAGSGAGAGSGAGAGSGVGVPGVGVPGAGAGSGAGAGSGAGAGSGAGAGSGAGAGSGAGAGSGVGVPGVGVPGAGAGSGAGAGSGAGAGSGAGAGSGAGAGSGAGAGSGVGVPGVGVPGAGAGSGAGAGSGAGAGSGAGAGSGAGAGSGAGAGSGVGVPGVGVPGAGAGSGAGAGSGAGAGSGAGAGSGAGAGSGAGAGSGVGVPGVGVPGAGAGSGAGAGSGAGAGSGAGAGSGAGAGSGAGAGSGVGVPGVGVPGAGAGSGAGAGSGAGAGSGAGAGSGAGAGSGAGAGSGVGVPGVGVPGAGAGSGAGAGSGAGAGSGAGAGSGAGAGSGAGAGSGVGVPGVGVPGAGAGSGAGAGSGAGAGSGAGAGSGAGAGSGAGAGSGVGVPGVGVPGAGAGSGAGAGSGAGAGSGAGAGSGAGAGSGAGAGSGVGVPGVGVPGAGAGSGAGAGSGAGAGSGAGAGSGAGAGSGAGAGSGVGVPGVGVPGAGAGSGAGAGSGAGAGSGAGAGSGAGAGSGAGAGSGVGVPGVGVPGAGAGSGAGAGSGAGAGSGAGAGSGAGAGSGAGAGSGVGVPGVGVPGAGAGSGAGAGSGAGAGSGAGAGSGAGAGSGAGAGSGVGVPGVGVPGAGAGSGAGAGSGAGAGSGAGAGSGAGAGSGAGAGSGVGVPGVGVPGAGAGSGAGAGSGAGAGSGAGAGSGAGAGSGAGAGSGVGVPGVGVPGAGAGSGAGAGSGAGAGSGAGAGSGAGAGSGAGAGSGVGVPGVGVPGAGAGSGAGAGSGAGAGSGAGAGSGAGAGSGAGAGSGVGVPGVGVPMDPGRYQDLRSHHHHHH

SEQ ID NO: 18 - protein, 2690 aa, Artificial Sequence
  ELP 1.1
MDPVVLQRRDWENPGVTQLNRLAAHPPFASDPMVPGVGVPGVGVPGVGVPGVGGAGAGSVPGVGVPGVGVPGVGVPGVGVPGVGVPGVGVPGVGVPGVGVPGVGVPGVGVPGVGVPGVGGAGAGSVPGVGVPGVGVPGVGVPGVGVPGVGVPGVGVPGVGVPGVGVPGVGVPGVGVPGVGVPGVGGAGAGSVPGVGVPGVGVPGVGVPGVGVPGVGVPGVGVPGVGVPGVGVPGVGVPGVGVPGVGVPGVGGAGAGSVPGVGVPGVGVPGVGVPGVGVPGVGVPGVGVPGVGVPGVGVPGVGVPGVGVPGVGVPGVGGAGAGSVPGVGVPGVGVPGVGVPGVGVPGVGVPGVGVPGVGVPGVGVPGVGVPGVGVPGVGVPGVGGAGAGSVPGVGVPGVGVPGVGVPGVGVPGVGVPGVGVPGVGVPGVGVPGVGVPGVGVPGVGVPGVGGAGAGSVPGVGVPGVGVPGVGVPGVGVPGVGVPGVGVPGVGVPGVGVPGVGVPGVGVPGVGVPGVGGAGAGSVPGVGVPGVGVPGVGVPGVGVPGVGVPGVGVPGVGVPGVGVPGVGVPGVGVPGVGVPGVGGAGAGSVPGVGVPGVGVPGVGVPGVGVPGVGVPGVGVPGVGVPGVGVPGVGVPGVGVPGVGVPGVGGAGAGSVPGVGVPGVGVPGVGVPGVGVPGVGVPGVGVPGVGVPGVGVPGVGVPGVGVPGVGVPGVGGAGAGSVPGVGVPGVGVPGVGVPGVGVPGVGVPGVGVPGVGVPGVGVPGVGVPGVGVPGVGVPGVGGAGAGSVPGVGVPGVGVPGVGVPGVGVPGVGVPGVGVPGVGVPGVGVPGVGVPGVGVPGVGVPGVGGAGAGSVPGVGVPGVGVPGVGVPGVGVPGVGVPGVGVPGVGVPGVGVPGVGVPGVGVPGVGVPGVGGAGAGSVPGVGVPGVGVPGVGVPGVGVPGVGVPGVGVPGVGVPGVGVPGVGVPGVGVPGVGVPGVGGAGAGSVPGVGVPGVGVPGVGVPGVGVPGVGVPGVGVPGVGVPGVGVPGVGVPGVGVPGVGVPGVGGAGAGSVPGVGVPGVGVPGVGVPGVGVPGVGVPGVGVPGVGVPGVGVPGVGVPGVGVPGVGVPGVGGAGAGSVPGVGVPGVGVPGVGVPGVGVPGVGVPGVGVPGVGVPGVGVPGVGVPGVGVPGVGVPGVGGAGAGSVPGVGVPGVGVPGVGVPGVGVPGVGVPGVGVPGVGVPGVGVPGVGVPGVGVPGVGVPGVGGAGAGSVPGVGVPGVGVPGVGVPGVGVPGVGVPGVGVPGVGVPGVGVPGVGVPGVGVPGVGVPGVGGAGAGSVPGVGVPGVGVPGVGVPGVGVPGVGVPGVGVPGVGVPGVGVPGVGVPGVGVPGVGVPGVGGAGAGSVPGVGVPGVGVPGVGVPGVGVPGVGVPGVGVPGVGVPGVGVPGVGVPGVGVPGVGVPGVGGAGAGSVPGVGVPGVGVPGVGVPGVGVPGVGVPGVGVPGVGVPGVGVPGVGVPGVGVPGVGVPGVGGAGAGSVPGVGVPGVGVPGVGVPGVGVPGVGVPGVGVPGVGVPGVGVPGVGVPGVGVPGVGVPGVGGAGAGSVPGVGVPGVGVPGVGVPGVGVPGVGVPGVGVPGVGVPGVGVPGVGVPGVGVPGVGVPGVGGAGAGSVPGVGVPGVGVPGVGVPGVGVPGVGVPGVGVPGVGVPGVGVPGVGVPGVGVPGVGVPGVGGAGAGSVPGVGVPGVGVPGVGVPGVGVPGVGVPGVGVPGVGVPGVGVPGVGVPGVGVPGVGVPGVGGAGAGSVPGVGVPGVGVPGVGVPGVGVPGVGVPGVGVPGVGVPGVGVPGVGVPGVGVPGVGVPGVGGAGAGSVPGVGVPGVGVPGVGVPGVGVPGVGVPGVGVPGVGVPGVGVPGVGVPGVGVPGVGVPGVGGAGAGSVPGVGVPGVGVPGVGVPGVGVPGVGVPGVGVPGVGVPGVGVPGVGVPGVGVPGVGVPGVGGAGAGSVPGVGVPGVGVPGVGVPGVGVPGVGVPGVGVPGVGVPGVGVPGVGVPGVGVPGVGVPGVGGAGAGSVPGVGVPGVGVPGVGVPGVGVPGVGVPGVGVPGVGVPGVGVPGVGVPGVGVPGVGVPGVGGAGAGSVPGVGVPGVGVPGVGVPGVGVPGVGVPGVGVPGVGVPGVGVPGVGVPGVGVPGVGVPGVGGAGAGSVPGVGVPGVGVPGVGVPGVGVPGVGVPGVGVPGVGVPGVGVPGVGVPGVGVPGVGVPGVGGAGAGSVPGVGVPGVGVPGVGVPGVGVPGVGVPGVGVPGVGVPGVGVPGVGVPGVGVPGVGVPGVGGAGAGSVPGVGVPGVGVPGVGVPGVGVPGVGVPGVGVPGVGVPGVGVPGVGVPGVGVPGVGVPGVGGAGAGSVPGVGVPGVGVPGVGVPGVGVPGVGVPGVGVPGVGVPGVGVPGVGVPGVGVPGVGVPGVGGAGAGSVPGVGVPGVGVPGVGVPGVGVPGVGVPGVGVPGVGVPGVGVPGVGVPGVGVPGVGVPGVGGAGAGSVPGVGVPGVGVPGVGVPGVGVPGVGVPGVGVPGVGVPGVGVPGVGVPGVGVPGVGVPGVGGAGAGSVPGVGVPGVGVPGVGVPGVGVPGVGVPGVGVPGVGVPGVGVPGVGVPGVGVPGVGVPGVGGAGAGSVPGVGVPGVGVPGVGVPGVGVPGVGVPGVGVPGVGVPGVGMDPGRYQDLRSHHHHHH

SEQ ID NO: 19 - protein, 1534 aa, Artificial Sequence
  SLP4.1.3
MDPVVLQRRDWENPGVTQLNRLAAHPPFASDPMGAGSGAGAGSGAGAGSGAGAGSGAGAGSGAGAGSGAGAGSGAGAGSGAGAGSGAGAGSGAGAGSGAGAGSGKGVPGKGVPGAGAGSGAGAGSGAGAGSGAGAGSGAGAGSGAGAGSGAGAGSGAGAGSGAGAGSGAGAGSGKGVPGKGVPGAGAGSGAGAGSGAGAGSGAGAGSGAGAGSGAGAGSGAGAGSGAGAGSGAGAGSGAGAGSGKGVPGKGVPGAGAGSGAGAGSGAGAGSGAGAGSGAGAGSGAGAGSGAGAGSGAGAGSGAGAGSGAGAGSGKGVPGKGVPGAGAGSGAGAGSGAGAGSGAGAGSGAGAGSGAGAGSGAGAGSGAGAGSGAGAGSGAGAGSGKGVPGKGVPGAGAGSGAGAGSGAGAGSGAGAGSGAGAGSGAGAGSGAGAGSGAGAGSGAGAGSGAGAGSGKGVPGKGVPGAGAGSGAGAGSGAGAGSGAGAGSGAGAGSGAGAGSGAGAGSGAGAGSGAGAGSGAGAGSGKGVPGKGVPGAGAGSGAGAGSGAGAGSGAGAGSGAGAGSGAGAGSGAGAGSGAGAGSGAGAGSGAGAGSGKGVPGKGVPGAGAGSGAGAGSGAGAGSGAGAGSGAGAGSGAGAGSGAGAGSGAGAGSGAGAGSGAGAGSGKGVPGKGVPGAGAGSGAGAGSGAGAGSGAGAGSGAGAGSGAGAGSGAGAGSGAGAGSGAGAGSGAGAGSGKGVPGKGVPGAGAGSGAGAGSGAGAGSGAGAGSGAGAGSGAGAGSGAGAGSGAGAGSGAGAGSGAGAGSGKGVPGKGVPGAGAGSGAGAGSGAGAGSGAGAGSGAGAGSGAGAGSGAGAGSGAGAGSGAGAGSGAGAGSGKGVPGKGVPGAGAGSGAGAGSGAGAGSGAGAGSGAGAGSGAGAGSGAGAGSGAGAGSGAGAGSGAGAGSGKGVPGKGVPGAGAGSGAGAGSGAGAGSGAGAGSGAGAGSGAGAGSGAGAGSGAGAGSGAGAGSGAGAGSGKGVPGKGVPGAGAGSGAGAGSGAGAGSGAGAGSGAGAGSGAGAGSGAGAGSGAGAGSGAGAGSGAGAGSGKGVPGKGVPGAGAGSGAGAGSGAGAGSGAGAGSGAGAGSGAGAGSGAGAGSGAGAGSGAGAGSGAGAGSGKGVPGKGVPGAGAGSGAGAGSGAGAGSGAGAGSGAGAGSGAGAGSGAGAGSGAGAGSGAGAGSGAGAGSGKGVPGKGVPGAGAGSGAGAGSGAGAGSGAGAGSGAGAGSGAGAGSGAGAGSGAGAGSGAGAGSGAGAGSGKGVPGKGVPGAGAGSGAGAGSGAGAGSGAGAGSGAGAGSGAGAGSGAGAGSGAGAGSGAGAGSGAGAGSGKGVPGKGVPGAGAGSGAGAGSGAGAGSGAGAGSGAGAGSGAGAGSGAGAGSGAGAGSGAGAGSGAGAGSGKGVPGKGVPGAGAGSGAGAGSGAGAGSGAGAGSGAGAGSGAGAGSGAGAGSGAGAGSGAGAGSGAGAGSGKGVPGKGVPGAGAMDPGRYQDLRSHHHHHH